European Patent Application EP 4 349 871 A1, published April 10, 2024. Title: 多肽及其用途. Applicant: 山西锦波生物医药股份有限公司. Application CN. The sequence listing filed with the application follows.

SEQUENCE LISTING (34 sequences)

SEQ ID NO: 1 - protein, 30 aa, synthetic construct
  REGION 1..30: note
GERGAPGFRGPAGPNGIPGEKGPAGERGAP

SEQ ID NO: 2 - protein, 9 aa, synthetic construct
  REGION 1..9: note = C
GAPGPCCGG

SEQ ID NO: 3 - protein, 489 aa, synthetic construct
  REGION 1..489: note = AT16
GERGAPGFRGPAGPNGIPGEKGPAGERGAPGERGAPGFRGPAGPNGIPGEKGPAGERGAPGERGAPGFRGPAGPNGIPGEKGPAGERGAPGERGAPGFRGPAGPNGIPGEKGPAGERGAPGERGAPGFRGPAGPNGIPGEKGPAGERGAPGERGAPGFRGPAGPNGIPGEKGPAGERGAPGERGAPGFRGPAGPNGIPGEKGPAGERGAPGERGAPGFRGPAGPNGIPGEKGPAGERGAPGERGAPGFRGPAGPNGIPGEKGPAGERGAPGERGAPGFRGPAGPNGIPGEKGPAGERGAPGERGAPGFRGPAGPNGIPGEKGPAGERGAPGERGAPGFRGPAGPNGIPGEKGPAGERGAPGERGAPGFRGPAGPNGIPGEKGPAGERGAPGERGAPGFRGPAGPNGIPGEKGPAGERGAPGERGAPGFRGPAGPNGIPGEKGPAGERGAPGERGAPGFRGPAGPNGIPGEKGPAGERGAPGAPGPCCGG

SEQ ID NO: 4 - DNA, 1467 bp, synthetic construct
  misc_feature 1..1467: note = AT16
  source 1..1467: mol_type = other DNA
ggagaaaggggggcgcctggctttcgtggtccggcgggtccgaatggcattccgggtgaaaagggtcctgccggtgagcgtggtgctccgggtgagcgcggcgctccgggtttccgcggtcccgcgggtccgaacggcatcccgggagaaaaaggcccagctggcgagcgcggtgcaccgggcgaacgtggtgccccgggcttccgtggcccagcgggtccgaacggtattccgggcgagaaaggtccggcaggtgaacgtggtgcgccaggcgagcgtggtgcgcctggtttcagaggcccagcaggcccaaatggcatccccggtgagaagggcccagccggtgagcgcggggcaccgggtgaacgtggcgcgccgggctttcgcggaccggcgggtccgaacggcatcccgggtgagaagggtccggctggcgagcgtggtgcgccgggtgaacgtggtgcaccgggattccgcggcccggcgggaccgaatggtattccgggtgagaagggtccggcgggcgaacgcggagcaccaggcgaacgcggcgctccgggctttcgcggtccggcgggtccgaatggtatcccgggcgagaagggtcctgccggtgagcgtggtgccccgggcgaacgtggcgctccgggttttcgtggtccggcgggtccgaacggcattccgggtgaaaagggcccagcgggtgagcgtggcgcgccaggcgagagaggtgccccgggttttcgtggcccggcgggtccgaacggcatcccgggtgagaaaggcccggcgggcgaacgtggtgcgccaggcgagagaggtgctccgggtttccgtggcccggctggtccgaacggtattccgggtgaaaagggcccggcgggcgagcgtggcgcgccgggtgagcgtggtgccccaggctttcgtggtccagctggtccgaacggtatcccgggtgaaaaaggtccggcgggtgagcgtggcgcgccgggtgaacgtggtgccccaggcttccgcgggccggcaggtcccaacggtatcccgggcgagaaaggtccggctggcgagcgaggtgccccgggcgaacgtggcgcgccgggcttccgcggtccggcaggcccgaacggtatcccgggcgagaaaggtccggcaggtgagcgtggtgcgccgggtgaacgcggcgctccgggttttcgtggcccggcaggcccaaatggcattccgggcgaaaaaggcccagcgggtgagcgtggtgccccgggtgagcgcggtgcgccgggtttccgcggtccggcgggtccgaatggtattccgggcgaaaaaggcccggcgggcgagcgtggcgctccgggcgaacgtggagcgccaggattccgcggcccggcaggaccgaacggcatcccgggagaaaagggcccggcgggtgaacgtggtgcaccgggagcgcctggtccgtgttgcggtggt

SEQ ID NO: 5 - protein, 498 aa, synthetic construct
  REGION 1..498: note = T16
GERGAPGFRGPAGPNGIPGEKGPAGERGAPGERGAPGFRGPAGPNGIPGEKGPAGERGAPGERGAPGFRGPAGPNGIPGEKGPAGERGAPGERGAPGFRGPAGPNGIPGEKGPAGERGAPRSGERGAPGFRGPAGPNGIPGEKGPAGERGAPGERGAPGFRGPAGPNGIPGEKGPAGERGAPGERGAPGFRGPAGPNGIPGEKGPAGERGAPGERGAPGFRGPAGPNGIPGEKGPAGERGAPRSGERGAPGFRGPAGPNGIPGEKGPAGERGAPGERGAPGFRGPAGPNGIPGEKGPAGERGAPGERGAPGFRGPAGPNGIPGEKGPAGERGAPGERGAPGFRGPAGPNGIPGEKGPAGERGAPRSGERGAPGFRGPAGPNGIPGEKGPAGERGAPGERGAPGFRGPAGPNGIPGEKGPAGERGAPGERGAPGFRGPAGPNGIPGEKGPAGERGAPGERGAPGFRGPAGPNGIPGEKGPAGERGAPRSGPPGPCCGGG

SEQ ID NO: 6 - protein, 480 aa, synthetic construct
  REGION 1..480: note = T16c
GERGAPGFRGPAGPNGIPGEKGPAGERGAPGERGAPGFRGPAGPNGIPGEKGPAGERGAPGERGAPGFRGPAGPNGIPGEKGPAGERGAPGERGAPGFRGPAGPNGIPGEKGPAGERGAPGERGAPGFRGPAGPNGIPGEKGPAGERGAPGERGAPGFRGPAGPNGIPGEKGPAGERGAPGERGAPGFRGPAGPNGIPGEKGPAGERGAPGERGAPGFRGPAGPNGIPGEKGPAGERGAPGERGAPGFRGPAGPNGIPGEKGPAGERGAPGERGAPGFRGPAGPNGIPGEKGPAGERGAPGERGAPGFRGPAGPNGIPGEKGPAGERGAPGERGAPGFRGPAGPNGIPGEKGPAGERGAPGERGAPGFRGPAGPNGIPGEKGPAGERGAPGERGAPGFRGPAGPNGIPGEKGPAGERGAPGERGAPGFRGPAGPNGIPGEKGPAGERGAPGERGAPGFRGPAGPNGIPGEKGPAGERGAP

SEQ ID NO: 7 - protein, 12 aa, synthetic construct
GPAGPNGIPGEK

SEQ ID NO: 8 - protein, 18 aa, synthetic construct
GPAGPNGIPGEKGPAGER

SEQ ID NO: 9 - protein, 18 aa, synthetic construct
GAPGFRGPAGPNGIPGEK

SEQ ID NO: 10 - protein, 24 aa, synthetic construct
GAPGFRGPAGPNGIPGEKGPAGER

SEQ ID NO: 11 - protein, 129 aa, synthetic construct
GERGAPGFRGPAGPNGIPGEKGPAGERGAPGERGAPGFRGPAGPNGIPGEKGPAGERGAPGERGAPGFRGPAGPNGIPGEKGPAGERGAPGERGAPGFRGPAGPNGIPGEKGPAGERGAPGAPGPCCGG

SEQ ID NO: 12 - DNA, 387 bp, synthetic construct
  source 1..387: mol_type = other DNA
ggagaaaggggggcgcctggctttcgtggtccggcgggtccgaatggcattccgggtgaaaagggtcctgccggtgagcgtggtgctccgggtgagcgcggcgctccgggtttccgcggtcccgcgggtccgaacggcatcccgggagaaaaaggcccagctggcgagcgcggtgcaccgggcgaacgtggtgccccgggcttccgtggcccagcgggtccgaacggtattccgggcgagaaaggtccggcaggtgaacgtggtgcgccaggcgagcgtggtgcgcctggtttcagaggcccagcaggcccaaatggcatccccggtgagaagggcccagccggtgagcgcggggcaccgggagcgcctggtccgtgttgcggtggt

SEQ ID NO: 13 - protein, 249 aa, synthetic construct
GERGAPGFRGPAGPNGIPGEKGPAGERGAPGERGAPGFRGPAGPNGIPGEKGPAGERGAPGERGAPGFRGPAGPNGIPGEKGPAGERGAPGERGAPGFRGPAGPNGIPGEKGPAGERGAPGERGAPGFRGPAGPNGIPGEKGPAGERGAPGERGAPGFRGPAGPNGIPGEKGPAGERGAPGERGAPGFRGPAGPNGIPGEKGPAGERGAPGERGAPGFRGPAGPNGIPGEKGPAGERGAPGAPGPCCGG

SEQ ID NO: 14 - DNA, 747 bp, synthetic construct
  source 1..747: mol_type = other DNA
ggagaaaggggggcgcctggctttcgtggtccggcgggtccgaatggcattccgggtgaaaagggtcctgccggtgagcgtggtgctccgggtgagcgcggcgctccgggtttccgcggtcccgcgggtccgaacggcatcccgggagaaaaaggcccagctggcgagcgcggtgcaccgggcgaacgtggtgccccgggcttccgtggcccagcgggtccgaacggtattccgggcgagaaaggtccggcaggtgaacgtggtgcgccaggcgagcgtggtgcgcctggtttcagaggcccagcaggcccaaatggcatccccggtgagaagggcccagccggtgagcgcggggcaccgggtgaacgtggcgcgccgggctttcgcggaccggcgggtccgaacggcatcccgggtgagaagggtccggctggcgagcgtggtgcgccgggtgaacgtggtgcaccgggattccgcggcccggcgggaccgaatggtattccgggtgagaagggtccggcgggcgaacgcggagcaccaggcgaacgcggcgctccgggctttcgcggtccggcgggtccgaatggtatcccgggcgagaagggtcctgccggtgagcgtggtgccccgggcgaacgtggcgctccgggttttcgtggtccggcgggtccgaacggcattccgggtgaaaagggcccagcgggtgagcgtggcgcgccaggagcgcctggtccgtgttgcggtggt

SEQ ID NO: 15 - protein, 369 aa, synthetic construct
GERGAPGFRGPAGPNGIPGEKGPAGERGAPGERGAPGFRGPAGPNGIPGEKGPAGERGAPGERGAPGFRGPAGPNGIPGEKGPAGERGAPGERGAPGFRGPAGPNGIPGEKGPAGERGAPGERGAPGFRGPAGPNGIPGEKGPAGERGAPGERGAPGFRGPAGPNGIPGEKGPAGERGAPGERGAPGFRGPAGPNGIPGEKGPAGERGAPGERGAPGFRGPAGPNGIPGEKGPAGERGAPGERGAPGFRGPAGPNGIPGEKGPAGERGAPGERGAPGFRGPAGPNGIPGEKGPAGERGAPGERGAPGFRGPAGPNGIPGEKGPAGERGAPGERGAPGFRGPAGPNGIPGEKGPAGERGAPGAPGPCCGG

SEQ ID NO: 16 - DNA, 1107 bp, synthetic construct
  source 1..1107: mol_type = other DNA
ggagaaaggggggcgcctggctttcgtggtccggcgggtccgaatggcattccgggtgaaaagggtcctgccggtgagcgtggtgctccgggtgagcgcggcgctccgggtttccgcggtcccgcgggtccgaacggcatcccgggagaaaaaggcccagctggcgagcgcggtgcaccgggcgaacgtggtgccccgggcttccgtggcccagcgggtccgaacggtattccgggcgagaaaggtccggcaggtgaacgtggtgcgccaggcgagcgtggtgcgcctggtttcagaggcccagcaggcccaaatggcatccccggtgagaagggcccagccggtgagcgcggggcaccgggtgaacgtggcgcgccgggctttcgcggaccggcgggtccgaacggcatcccgggtgagaagggtccggctggcgagcgtggtgcgccgggtgaacgtggtgcaccgggattccgcggcccggcgggaccgaatggtattccgggtgagaagggtccggcgggcgaacgcggagcaccaggcgaacgcggcgctccgggctttcgcggtccggcgggtccgaatggtatcccgggcgagaagggtcctgccggtgagcgtggtgccccgggcgaacgtggcgctccgggttttcgtggtccggcgggtccgaacggcattccgggtgaaaagggcccagcgggtgagcgtggcgcgccaggcgagagaggtgccccgggttttcgtggcccggcgggtccgaacggcatcccgggtgagaaaggcccggcgggcgaacgtggtgcgccaggcgagagaggtgctccgggtttccgtggcccggctggtccgaacggtattccgggtgaaaagggcccggcgggcgagcgtggcgcgccgggtgagcgtggtgccccaggctttcgtggtccagctggtccgaacggtatcccgggtgaaaaaggtccggcgggtgagcgtggcgcgccgggtgaacgtggtgccccaggcttccgcgggccggcaggtcccaacggtatcccgggcgagaaaggtccggctggcgagcgaggtgccccgggagcgcctggtccgtgttgcggtggt

SEQ ID NO: 17 - protein, 609 aa, synthetic construct
GERGAPGFRGPAGPNGIPGEKGPAGERGAPGERGAPGFRGPAGPNGIPGEKGPAGERGAPGERGAPGFRGPAGPNGIPGEKGPAGERGAPGERGAPGFRGPAGPNGIPGEKGPAGERGAPGERGAPGFRGPAGPNGIPGEKGPAGERGAPGERGAPGFRGPAGPNGIPGEKGPAGERGAPGERGAPGFRGPAGPNGIPGEKGPAGERGAPGERGAPGFRGPAGPNGIPGEKGPAGERGAPGERGAPGFRGPAGPNGIPGEKGPAGERGAPGERGAPGFRGPAGPNGIPGEKGPAGERGAPGERGAPGFRGPAGPNGIPGEKGPAGERGAPGERGAPGFRGPAGPNGIPGEKGPAGERGAPGERGAPGFRGPAGPNGIPGEKGPAGERGAPGERGAPGFRGPAGPNGIPGEKGPAGERGAPGERGAPGFRGPAGPNGIPGEKGPAGERGAPGERGAPGFRGPAGPNGIPGEKGPAGERGAPGERGAPGFRGPAGPNGIPGEKGPAGERGAPGERGAPGFRGPAGPNGIPGEKGPAGERGAPGERGAPGFRGPAGPNGIPGEKGPAGERGAPGERGAPGFRGPAGPNGIPGEKGPAGERGAPGAPGPCCGG

SEQ ID NO: 18 - DNA, 1827 bp, synthetic construct
  source 1..1827: mol_type = other DNA
ggagaaaggggggcgcctggctttcgtggtccggcgggtccgaatggcattccgggtgaaaagggtcctgccggtgagcgtggtgctccgggtgagcgcggcgctccgggtttccgcggtcccgcgggtccgaacggcatcccgggagaaaaaggcccagctggcgagcgcggtgcaccgggcgaacgtggtgccccgggcttccgtggcccagcgggtccgaacggtattccgggcgagaaaggtccggcaggtgaacgtggtgcgccaggcgagcgtggtgcgcctggtttcagaggcccagcaggcccaaatggcatccccggtgagaagggcccagccggtgagcgcggggcaccgggtgaacgtggcgcgccgggctttcgcggaccggcgggtccgaacggcatcccgggtgagaagggtccggctggcgagcgtggtgcgccgggtgaacgtggtgcaccgggattccgcggcccggcgggaccgaatggtattccgggtgagaagggtccggcgggcgaacgcggagcaccaggcgaacgcggcgctccgggctttcgcggtccggcgggtccgaatggtatcccgggcgagaagggtcctgccggtgagcgtggtgccccgggcgaacgtggcgctccgggttttcgtggtccggcgggtccgaacggcattccgggtgaaaagggcccagcgggtgagcgtggcgcgccaggcgagagaggtgccccgggttttcgtggcccggcgggtccgaacggcatcccgggtgagaaaggcccggcgggcgaacgtggtgcgccaggcgagagaggtgctccgggtttccgtggcccggctggtccgaacggtattccgggtgaaaagggcccggcgggcgagcgtggcgcgccgggtgagcgtggtgccccaggctttcgtggtccagctggtccgaacggtatcccgggtgaaaaaggtccggcgggtgagcgtggcgcgccgggtgaacgtggtgccccaggcttccgcgggccggcaggtcccaacggtatcccgggcgagaaaggtccggctggcgagcgaggtgccccgggcgaacgtggcgcgccgggcttccgcggtccggcaggcccgaacggtatcccgggcgagaaaggtccggcaggtgagcgtggtgcgccgggtgaacgcggcgctccgggttttcgtggcccggcaggcccaaatggcattccgggcgaaaaaggcccagcgggtgagcgtggtgccccgggtgagcgcggtgcgccgggtttccgcggtccggcgggtccgaatggtattccgggcgaaaaaggcccggcgggcgagcgtggcgctccgggcgaacgtggagcgccaggattccgcggcccggcaggaccgaacggcatcccgggagaaaagggcccggcgggtgaacgtggtgcaccgggagaaaggggggcgcctggctttcgtggtccggcgggtccgaatggcattccgggtgaaaagggtcctgccggtgagcgtggtgctccgggtgagcgcggcgctccgggtttccgcggtcccgcgggtccgaacggcatcccgggagaaaaaggcccagctggcgagcgcggtgcaccgggcgaacgtggtgccccgggcttccgtggcccagcgggtccgaacggtattccgggcgagaaaggtccggcaggtgaacgtggtgcgccaggcgagcgtggtgcgcctggtttcagaggcccagcaggcccaaatggcatccccggtgagaagggcccagccggtgagcgcggggcaccgggagcgcctggtccgtgttgcggtggt

SEQ ID NO: 19 - protein, 8 aa, synthetic construct
GPAGERGA

SEQ ID NO: 20 - protein, 12 aa, synthetic construct
GFRGPAGPNGIP

SEQ ID NO: 21 - protein, 15 aa, synthetic construct
GERGAPGERGAPGFR

SEQ ID NO: 22 - protein, 21 aa, synthetic construct
EKGPAGERGAPGERGAPGFRG

SEQ ID NO: 23 - protein, 10 aa, synthetic construct
GPNGIPGEKG

SEQ ID NO: 24 - protein, 13 aa, synthetic construct
KGPAGERGAPGER

SEQ ID NO: 25 - protein, 16 aa, synthetic construct
PAGPNGIPGEKGPAGE

SEQ ID NO: 26 - protein, 22 aa, synthetic construct
AGPNGIPGEKGPAGERGAPGER

SEQ ID NO: 27 - protein, 10 aa, synthetic construct
ERGAPGFRGP

SEQ ID NO: 28 - protein, 13 aa, synthetic construct
RGAPGERGAPGFR

SEQ ID NO: 29 - protein, 15 aa, synthetic construct
GPAGPNGIPGEKGPA

SEQ ID NO: 30 - protein, 23 aa, synthetic construct
NGIPGEKGPAGERGAPGERGAPG

SEQ ID NO: 31 - protein, 10 aa, synthetic construct
PAGPNGIPGE

SEQ ID NO: 32 - protein, 14 aa, synthetic construct
GFRGPAGPNGIPGE

SEQ ID NO: 33 - protein, 18 aa, synthetic construct
RGAPGERGAPGFRGPAGP

SEQ ID NO: 34 - protein, 24 aa, synthetic construct
PGERGAPGFRGPAGPNGIPGEKGP